European Patent Application EP 4 796 124 A1, published August 26, 2026. Title: Novel chimeric T cell receptor construct for enhanced immune cell-based immunotherapy. Applicant: MEDIGENE IMMUNOTHERAPIES GMBH. Application EP. The sequence listing filed with the application follows.

SEQUENCE LISTING (94 sequences)

SEQ ID NO: 1 - protein, 21 aa, Homo sapiens
  source 1..21: note = NKp46 signal sequence
MSSTLPALLCVGLCLSQRISA

SEQ ID NO: 2 - protein, 18 aa, Homo sapiens
  source 1..18: note = NKp30 signal sequence
MAWMLLLILIMVHPGSCA

SEQ ID NO: 3 - protein, 21 aa, Homo sapiens
  source 1..21: note = NKp44 signal sequence
MAWRALHPLLLLLLLFPGSQA

SEQ ID NO: 4 - protein, 21 aa, Homo sapiens
  source 1..21: note = TCR alpha signal sequence
MKSLRVLLVILWLQLSWVWSQ

SEQ ID NO: 5 - protein, 19 aa, Homo sapiens
  source 1..19: note = TCR beta signal sequence
MGSWTLCCVSLCILVAKHT

SEQ ID NO: 6 - protein, 134 aa, Homo sapiens
  source 1..134: note = CD3 zeta sequence
LCYLLDGILFIYGVILTALFLRVKFSRSADAPAYQQGQNQLYNELNLGRREEYDVLDKRRGRDPEMGGKPQRRKNPQEGLYNELQKDKMAEAYSEIGMKGERRRGKGHDGLYQGLSTATKDTYDALHMQALPPR

SEQ ID NO: 7 - protein, 134 aa, Homo sapiens; identical to SEQ ID NO: 6
  source 1..134: note = DAP10 signaling domain sequence

SEQ ID NO: 8 - protein, 4 aa, synthetic construct
  source 1..4: note = linker sequence 1
APAP

SEQ ID NO: 9 - protein, 4 aa, synthetic construct
  source 1..4: note = linker sequence 2
ESGS

SEQ ID NO: 10 - protein, 4 aa, synthetic construct
  source 1..4: note = linker sequence 3
GGGS

SEQ ID NO: 11 - protein, 5 aa, synthetic construct
  source 1..5: note = linker sequence 4
GGGGS

SEQ ID NO: 12 - protein, 6 aa, synthetic construct
  source 1..6: note = linker sequence 5
GSGGSG

SEQ ID NO: 13 - protein, 6 aa, Homo sapiens
  source 1..6: note = NYESO1 TCR alpha CDR1 sequence
DRGSQS

SEQ ID NO: 14 - protein, 6 aa, Homo sapiens
  source 1..6: note = NYESO1 TCR alpha CDR2 sequence
IYSNGD

SEQ ID NO: 15 - protein, 7 aa, Homo sapiens
  source 1..7: note = NYESO1 TCR alpha CDR3 sequence
AADDKII

SEQ ID NO: 16 - protein, 5 aa, Homo sapiens
  source 1..5: note = NYESO1 TCR beta CDR1 sequence
SGHDY

SEQ ID NO: 17 - protein, 6 aa, Homo sapiens
  source 1..6: note = NYESO1 TCR beta CDR2 sequence
FNNNVP

SEQ ID NO: 18 - protein, 10 aa, Homo sapiens
  source 1..10: note = NYESO1 TCR beta CDR3 sequence
ASSRGGSGYT

SEQ ID NO: 19 - protein, 108 aa, Homo sapiens
  source 1..108: note = NYESO1 V alpha sequence
QKEVEQNSGPLSVPEGAIASLNCTYSDRGSQSFFWYRQYSGKSPELIMFIYSNGDKEDGRFTAQLNKASQYVSLLIRDSQPSDSATYLCAADDKIIFGKGTRLHILPN

SEQ ID NO: 20 - protein, 112 aa, Homo sapiens
  source 1..112: note = NYESO1 V beta sequence
DAGVIQSPRHEVTEMGQEVTLRCKPISGHDYLFWYRQTMMRGLELLIYFNNNVPIDDSGMPEDRFSAKMPNASFSTLKIQPSEPRDSAVYFCASSRGGSGYTFGSGTRLTVV

SEQ ID NO: 21 - protein, 115 aa, Homo sapiens
  source 1..115: note = C alpha sequence
IQNPDPAVYQLRDSKSSDKSVCLFTDFDSQTNVSQSKDSDVYITDKCVLDMRSMDFKSNSAVAWSNKSDFACANAFNNSIIPEDTFFPSSDVPCDVKLVEKSFETDTNLNFQNLS

SEQ ID NO: 22 - protein, 145 aa, Homo sapiens
  source 1..145: note = C beta sequence
EDLNKVFPPEVAVFEPSKAEIAHTQKATLVCLATGFFPDHVELSWWVNGKEVHSGVCTDPQPLKEQPALNDSRYCLSSRLRVSATFWQNPRNHFRCQVQFYGLSENDEWTQDRAKPVTQIVSAEAWGRADCGITSASYHQGVLSA

SEQ ID NO: 23 - protein, 160 aa, synthetic construct
  source 1..160: note = C beta sequence with 9-mer epitope tag
EDLNKVFPPEVAVFEPSKAEIAHTQKATLVCLATGFFPDHVELSWWVNGKEVHSGVCTDPQPLKEQPALNDGSGGEVPKDRFSGSGSRYCLSSRLRVSATFWQNPRNHFRCQVQFYGLSENDEWTQDRAKPVTQIVSAEAWGRADCGITSASYHQGVLSA

SEQ ID NO: 24 - protein, 356 aa, synthetic construct
  source 1..356: note = Fusion protein NYESO1 TCR alpha chain and CD3 zeta chain sequence
QKEVEQNSGPLSVPEGAIASLNCTYSDRGSQSFFWYRQYSGKSPELIMFIYSNGDKEDGRFTAQLNKASQYVSLLIRDSQPSDSATYLCAADDKIIFGKGTRLHILPNIQNPDPAVYQLRDSKSSDKSVCLFTDFDSQTNVSQSKDSDVYITDKCVLDMRSMDFKSNSAVAWSNKSDFACANAFNNSIIPEDTFFPSSDVPCDVKLVEKSFETDTNLNFQNLSLCYLLDGILFIYGVILTALFLRVKFSRSADAPAYQQGQNQLYNELNLGRREEYDVLDKRRGRDPEMGGKPQRRKNPQEGLYNELQKDKMAEAYSEIGMKGERRRGKGHDGLYQGLSTATKDTYDALHMQALPP

SEQ ID NO: 25 - protein, 391 aa, synthetic construct
  source 1..391: note = Fusion protein NYESO1 TCR beta chain and CD3 zeta chain sequence
DAGVIQSPRHEVTEMGQEVTLRCKPISGHDYLFWYRQTMMRGLELLIYFNNNVPIDDSGMPEDRFSAKMPNASFSTLKIQPSEPRDSAVYFCASSRGGSGYTFGSGTRLTVVEDLNKVFPPEVAVFEPSKAEIAHTQKATLVCLATGFFPDHVELSWWVNGKEVHSGVCTDPQPLKEQPALNDSRYCLSSRLRVSATFWQNPRNHFRCQVQFYGLSENDEWTQDRAKPVTQIVSAEAWGRADCGITSASYHQGVLSALCYLLDGILFIYGVILTALFLRVKFSRSADAPAYQQGQNQLYNELNLGRREEYDVLDKRRGRDPEMGGKPQRRKNPQEGLYNELQKDKMAEAYSEIGMKGERRRGKGHDGLYQGLSTATKDTYDALHMQALPPR

SEQ ID NO: 26 - protein, 406 aa, synthetic construct
  source 1..406: note = 27: Fusion protein NYESO1 TCR beta chain and CD3 zeta chain sequence (no signal sequence; with 9-mer epitope tag)
DAGVIQSPRHEVTEMGQEVTLRCKPISGHDYLFWYRQTMMRGLELLIYFNNNVPIDDSGMPEDRFSAKMPNASFSTLKIQPSEPRDSAVYFCASSRGGSGYTFGSGTRLTVVEDLNKVFPPEVAVFEPSKAEIAHTQKATLVCLATGFFPDHVELSWWVNGKEVHSGVCTDPQPLKEQPALNDGSGGEVPKDRFSGSGSRYCLSSRLRVSATFWQNPRNHFRCQVQFYGLSENDEWTQDRAKPVTQIVSAEAWGRADCGITSASYHQGVLSALCYLLDGILFIYGVILTALFLRVKFSRSADAPAYQQGQNQLYNELNLGRREEYDVLDKRRGRDPEMGGKPQRRKNPQEGLYNELQKDKMAEAYSEIGMKGERRRGKGHDGLYQGLSTATKDTYDALHMQALPPR

SEQ ID NO: 27 - protein, 9 aa, synthetic construct
  source 1..9: note = 9-mer epitope tag
GEVPKDRFS

SEQ ID NO: 28 - protein, 6 aa, Homo sapiens
  source 1..6: note = KRASG12V-TCR6-TCR alpha CDR1 sequence
NSAFQY

SEQ ID NO: 29 - protein, 6 aa, Homo sapiens
  source 1..6: note = KRASG12V-TCR6-TCR alpha CDR2 sequence
TYSSGN

SEQ ID NO: 30 - protein, 10 aa, Homo sapiens
  source 1..10: note = KRASG12V-TCR6-TCR alpha CDR3 sequence
AMSARNNDMR

SEQ ID NO: 31 - protein, 5 aa, Homo sapiens
  source 1..5: note = KRASG12V-TCR6-TCR beta CDR1 sequence
SNHLY

SEQ ID NO: 32 - protein, 6 aa, Homo sapiens
  source 1..6: note = KRASG12V-TCR6-TCR beta CDR2 sequence
FYNNEI

SEQ ID NO: 33 - protein, 11 aa, Homo sapiens
  source 1..11: note = KRASG12V-TCR6-TCR beta CDR3 sequence
ARSGTSTGELF

SEQ ID NO: 34 - protein, 111 aa, Homo sapiens
  source 1..111: note = KRASG12V-TCR6-V alpha sequence (no signal sequence)
QKEVEQDPGPLSVPEGAIVSLNCTYSNSAFQYFMWYRQYSRKGPELLMYTYSSGNKEDGRFTAQVDKSSKYISLFIRDSQPSDSATYLCAMSARNNDMRFGAGTRLTVKPN

SEQ ID NO: 35 - protein, 113 aa, Homo sapiens
  source 1..113: note = KRASG12V-TCR6-V beta sequence (no signal sequence)
EPEVTQTPSHQVTQMGQEVILRCVPISNHLYFYWYRQILGQKVEFLVSFYNNEISEKSEIFDDQFSVERPDGSNFTLKIRSTKLEDSAMYFCARSGTSTGELFFGEGSRLTVL

SEQ ID NO: 36 - protein, 360 aa, synthetic construct
  source 1..360: note = Fusion protein KRASG12V-TCR6-TCR alpha chain and CD3 zeta chain sequence (no signal sequence)
QKEVEQDPGPLSVPEGAIVSLNCTYSNSAFQYFMWYRQYSRKGPELLMYTYSSGNKEDGRFTAQVDKSSKYISLFIRDSQPSDSATYLCAMSARNNDMRFGAGTRLTVKPNIQNPDPAVYQLRDSKSSDKSVCLFTDFDSQTNVSQSKDSDVYITDKCVLDMRSMDFKSNSAVAWSNKSDFACANAFNNSIIPEDTFFPSSDVPCDVKLVEKSFETDTNLNFQNLSLCYLLDGILFIYGVILTALFLRVKFSRSADAPAYQQGQNQLYNELNLGRREEYDVLDKRRGRDPEMGGKPQRRKNPQEGLYNELQKDKMAEAYSEIGMKGERRRGKGHDGLYQGLSTATKDTYDALHMQALPPR

SEQ ID NO: 37 - protein, 398 aa, synthetic construct
  source 1..398: note = Fusion protein KRASG12V-TCR6-TCR beta chain and CD3 zeta chain sequence (no signal sequence)
EPEVTQTPSHQVTQMGQEVILRCVPISNHLYFYWYRQILGQKVEFLVSFYNNEISEKSEIFDDQFSVERPDGSNFTLKIRSTKLEDSAMYFCARSGTSTGELFFGEGSRLTVLEDLNKVFPPEVAVFEPSKAEIAHTQKATLVCLATGFFPDHVELSWWVNGKEVHSGVCTDPQPLKEQPALNDGSGGSGSRYCLSSRLRVSATFWQNPRNHFRCQVQFYGLSENDEWTQDRAKPVTQIVSAEAWGRADCGITSASYHQGVLSALCYLLDGILFIYGVILTALFLRVKFSRSADAPAYQQGQNQLYNELNLGRREEYDVLDKRRGRDPEMGGKPQRRKNPQEGLYNELQKDKMAEAYSEIGMKGERRRGKGHDGLYQGLSTATKDTYDALHMQALPPR

SEQ ID NO: 38 - protein, 407 aa, synthetic construct
  source 1..407: note = Fusion protein KRASG12V-TCR6-TCR beta chain and CD3 zeta chain sequence (no signal sequence; with epitope tag)
EPEVTQTPSHQVTQMGQEVILRCVPISNHLYFYWYRQILGQKVEFLVSFYNNEISEKSEIFDDQFSVERPDGSNFTLKIRSTKLEDSAMYFCARSGTSTGELFFGEGSRLTVLEDLNKVFPPEVAVFEPSKAEIAHTQKATLVCLATGFFPDHVELSWWVNGKEVHSGVCTDPQPLKEQPALNDGSGGEVPKDRFSGSGSRYCLSSRLRVSATFWQNPRNHFRCQVQFYGLSENDEWTQDRAKPVTQIVSAEAWGRADCGITSASYHQGVLSALCYLLDGILFIYGVILTALFLRVKFSRSADAPAYQQGQNQLYNELNLGRREEYDVLDKRRGRDPEMGGKPQRRKNPQEGLYNELQKDKMAEAYSEIGMKGERRRGKGHDGLYQGLSTATKDTYDALHMQALPPR

SEQ ID NO: 39 - protein, 6 aa, Homo sapiens
  source 1..6: note = PRAME-VLD-TCR alpha CDR1 sequence
VSGLRG

SEQ ID NO: 40 - protein, 8 aa, Homo sapiens
  source 1..8: note = PRAME-VLD-TCR alpha CDR2 sequence
LYSAGEEE

SEQ ID NO: 41 - protein, 13 aa, Homo sapiens
  source 1..13: note = PRAME-VLD-TCR alpha CDR3 sequence
AVHSTAQAGTALI

SEQ ID NO: 42 - protein, 5 aa, Homo sapiens
  source 1..5: note = PRAME-VLD-TCR beta CDR1 sequence
SGDLS

SEQ ID NO: 43 - protein, 6 aa, Homo sapiens
  source 1..6: note = PRAME-VLD-TCR beta CDR2 sequence
YYNGEE

SEQ ID NO: 44 - protein, 14 aa, Homo sapiens
  source 1..14: note = PRAME-VLD-TCR beta CDR3 sequence
ASSTHRGQTNYGYT

SEQ ID NO: 45 - protein, 113 aa, Homo sapiens
  source 1..113: note = PRAME-VLD-V alpha sequence (no signal sequence)
EDQVTQSPEALRLQEGESSSLNCSYTVSGLRGLFWYRQDPGKGPEFLFTLYSAGEEKEKERLKATLTKKESFLHITAPKPEDSATYLCAVHSTAQAGTALIFGKGTTLSVSSN

SEQ ID NO: 46 - protein, 115 aa, Homo sapiens
  source 1..115: note = PRAME-VLD-V beta sequence (no signal sequence)
DSGVTQTPKHLITATGQRVTLRCSPRSGDLSVYWYQQSLDQGLQFLIQYYNGEERAKGNILERFSAQQFPDLHSELNLSSLELGDSALYFCASSTHRGQTNYGYTFGSGTRLTVV

SEQ ID NO: 47 - protein, 362 aa, synthetic construct
  source 1..362: note = Fusion protein PRAME-VLD-TCR alpha chain and CD3 zeta chain sequence (no signal sequence)
EDQVTQSPEALRLQEGESSSLNCSYTVSGLRGLFWYRQDPGKGPEFLFTLYSAGEEKEKERLKATLTKKESFLHITAPKPEDSATYLCAVHSTAQAGTALIFGKGTTLSVSSNIQNPDPAVYQLRDSKSSDKSVCLFTDFDSQTNVSQSKDSDVYITDKCVLDMRSMDFKSNSAVAWSNKSDFACANAFNNSIIPEDTFFPSSDVPCDVKLVEKSFETDTNLNFQNLSLCYLLDGILFIYGVILTALFLRVKFSRSADAPAYQQGQNQLYNELNLGRREEYDVLDKRRGRDPEMGGKPQRRKNPQEGLYNELQKDKMAEAYSEIGMKGERRRGKGHDGLYQGLSTATKDTYDALHMQALPPR

SEQ ID NO: 48 - protein, 394 aa, synthetic construct
  source 1..394: note = Fusion protein PRAME-VLD-TCR beta chain and CD3 zeta chain sequence (no signal sequence)
DSGVTQTPKHLITATGQRVTLRCSPRSGDLSVYWYQQSLDQGLQFLIQYYNGEERAKGNILERFSAQQFPDLHSELNLSSLELGDSALYFCASSTHRGQTNYGYTFGSGTRLTVVEDLNKVFPPEVAVFEPSKAEIAHTQKATLVCLATGFFPDHVELSWWVNGKEVHSGVCTDPQPLKEQPALNDSRYCLSSRLRVSATFWQNPRNHFRCQVQFYGLSENDEWTQDRAKPVTQIVSAEAWGRADCGITSASYHQGVLSALCYLLDGILFIYGVILTALFLRVKFSRSADAPAYQQGQNQLYNELNLGRREEYDVLDKRRGRDPEMGGKPQRRKNPQEGLYNELQKDKMAEAYSEIGMKGERRRGKGHDGLYQGLSTATKDTYDALHMQALPPR

SEQ ID NO: 49 - protein, 32 aa, Homo sapiens
  source 1..32: note = Signal sequence CD79A
MPGGPGVLQALPATIFLLFLLSAVYLGPGCQA

SEQ ID NO: 50 - protein, 28 aa, Homo sapiens
  source 1..28: note = Signal sequence CD79B
MARLALSPVPSHWMVALLLLLSAEPVPA

SEQ ID NO: 51 - protein, 19 aa, Homo sapiens
  source 1..19: note = Signal sequence CD14
MERASCLLLLLLPLVHVSA

SEQ ID NO: 52 - protein, 20 aa, Homo sapiens
  source 1..20: note = Signal sequence CD40
MVRLPLQCVLWGCLLTAVHP

SEQ ID NO: 53 - protein, 16 aa, Homo sapiens
  source 1..16: note = Signal sequence CD11b
MALRVLLLTALTLCHG

SEQ ID NO: 54 - protein, 15 aa, Homo sapiens
  source 1..15: note = Signal sequence CD64
MWFLTTLLLWVPVDG

SEQ ID NO: 55 - protein, 409 aa, synthetic construct
  source 1..409: note = Fusion protein PRAME-VLD-TCR beta chain and CD3 zeta chain sequence (no signal sequence; with 9-mer epitope tag)
DSGVTQTPKHLITATGQRVTLRCSPRSGDLSVYWYQQSLDQGLQFLIQYYNGEERAKGNILERFSAQQFPDLHSELNLSSLELGDSALYFCASSTHRGQTNYGYTFGSGTRLTVVEDLNKVFPPEVAVFEPSKAEIAHTQKATLVCLATGFFPDHVELSWWVNGKEVHSGVCTDPQPLKEQPALNDGSGGEVPKDRFSGSGSRYCLSSRLRVSATFWQNPRNHFRCQVQFYGLSENDEWTQDRAKPVTQIVSAEAWGRADCGITSASYHQGVLSALCYLLDGILFIYGVILTALFLRVKFSRSADAPAYQQGQNQLYNELNLGRREEYDVLDKRRGRDPEMGGKPQRRKNPQEGLYNELQKDKMAEAYSEIGMKGERRRGKGHDGLYQGLSTATKDTYDALHMQALPPR

SEQ ID NO: 56 - protein, 427 aa, synthetic construct
  source 1..427: note = Fusion protein NYESO1 TCR beta chain and CD3 zeta chain sequence (NKp46 signal sequence, with 9-mer epitope tag)
MSSTLPALLCVGLCLSQRISADAGVIQSPRHEVTEMGQEVTLRCKPISGHDYLFWYRQTMMRGLELLIYFNNNVPIDDSGMPEDRFSAKMPNASFSTLKIQPSEPRDSAVYFCASSRGGSGYTFGSGTRLTVVEDLNKVFPPEVAVFEPSKAEIAHTQKATLVCLATGFFPDHVELSWWVNGKEVHSGVCTDPQPLKEQPALNDGSGGEVPKDRFSGSGSRYCLSSRLRVSATFWQNPRNHFRCQVQFYGLSENDEWTQDRAKPVTQIVSAEAWGRADCGITSASYHQGVLSALCYLLDGILFIYGVILTALFLRVKFSRSADAPAYQQGQNQLYNELNLGRREEYDVLDKRRGRDPEMGGKPQRRKNPQEGLYNELQKDKMAEAYSEIGMKGERRRGKGHDGLYQGLSTATKDTYDALHMQALPPR

SEQ ID NO: 57 - protein, 378 aa, synthetic construct
  source 1..378: note = Fusion protein NYESO1 TCR alpha chain and CD3 zeta chain sequence (NKp46 signal sequence)
MSSTLPALLCVGLCLSQRISAQKEVEQNSGPLSVPEGAIASLNCTYSDRGSQSFFWYRQYSGKSPELIMFIYSNGDKEDGRFTAQLNKASQYVSLLIRDSQPSDSATYLCAADDKIIFGKGTRLHILPNIQNPDPAVYQLRDSKSSDKSVCLFTDFDSQTNVSQSKDSDVYITDKCVLDMRSMDFKSNSAVAWSNKSDFACANAFNNSIIPEDTFFPSSDVPCDVKLVEKSFETDTNLNFQNLSLCYLLDGILFIYGVILTALFLRVKFSRSADAPAYQQGQNQLYNELNLGRREEYDVLDKRRGRDPEMGGKPQRRKNPQEGLYNELQKDKMAEAYSEIGMKGERRRGKGHDGLYQGLSTATKDTYDALHMQALPPR

SEQ ID NO: 58 - protein, 454 aa, synthetic construct
  source 1..454: note = Fusion protein NYESO1 TCR beta chain, CD3 zeta chain and DAP10 sequence (NKp46 signal se-quence, with 9-mer epitope tag)
MSSTLPALLCVGLCLSQRISADAGVIQSPRHEVTEMGQEVTLRCKPISGHDYLFWYRQTMMRGLELLIYFNNNVPIDDSGMPEDRFSAKMPNASFSTLKIQPSEPRDSAVYFCASSRGGSGYTFGSGTRLTVVEDLNKVFPPEVAVFEPSKAEIAHTQKATLVCLATGFFPDHVELSWWVNGKEVHSGVCTDPQPLKEQPALNDGSGGEVPKDRFSGSGSRYCLSSRLRVSATFWQNPRNHFRCQVQFYGLSENDEWTQDRAKPVTQIVSAEAWGRADCGITSASYHQGVLSALCYLLDGILFIYGVILTALFLRVKFSRSADAPAYQQGQNQLYNELNLGRREEYDVLDKRRGRDPEMGGKPQRRKNPQEGLYNELQKDKMAEAYSEIGMKGERRRGKGHDGLYQGLSTATKDTYDALHMQALPPRGGSLCARPRRSPAQEDGKVYINMPGRG

SEQ ID NO: 59 - protein, 405 aa, synthetic construct
  source 1..405: note = Fusion protein NYESO1 TCR alpha chain, CD3 zeta chain and DAP10 sequence (NKp46 signal sequence)
MSSTLPALLCVGLCLSQRISAQKEVEQNSGPLSVPEGAIASLNCTYSDRGSQSFFWYRQYSGKSPELIMFIYSNGDKEDGRFTAQLNKASQYVSLLIRDSQPSDSATYLCAADDKIIFGKGTRLHILPNIQNPDPAVYQLRDSKSSDKSVCLFTDFDSQTNVSQSKDSDVYITDKCVLDMRSMDFKSNSAVAWSNKSDFACANAFNNSIIPEDTFFPSSDVPCDVKLVEKSFETDTNLNFQNLSLCYLLDGILFIYGVILTALFLRVKFSRSADAPAYQQGQNQLYNELNLGRREEYDVLDKRRGRDPEMGGKPQRRKNPQEGLYNELQKDKMAEAYSEIGMKGERRRGKGHDGLYQGLSTATKDTYDALHMQALPPRGGSLCARPRRSPAQEDGKVYINMPGRG

SEQ ID NO: 60 - protein, 424 aa, synthetic construct
  source 1..424: note = Fusion protein NYESO1 TCR beta chain and CD3 zeta chain sequence (NKp30 signal sequence, with 9-mer epitope tag)
MAWMLLLILIMVHPGSCADAGVIQSPRHEVTEMGQEVTLRCKPISGHDYLFWYRQTMMRGLELLIYFNNNVPIDDSGMPEDRFSAKMPNASFSTLKIQPSEPRDSAVYFCASSRGGSGYTFGSGTRLTVVEDLNKVFPPEVAVFEPSKAEIAHTQKATLVCLATGFFPDHVELSWWVNGKEVHSGVCTDPQPLKEQPALNDGSGGEVPKDRFSGSGSRYCLSSRLRVSATFWQNPRNHFRCQVQFYGLSENDEWTQDRAKPVTQIVSAEAWGRADCGITSASYHQGVLSALCYLLDGILFIYGVILTALFLRVKFSRSADAPAYQQGQNQLYNELNLGRREEYDVLDKRRGRDPEMGGKPQRRKNPQEGLYNELQKDKMAEAYSEIGMKGERRRGKGHDGLYQGLSTATKDTYDALHMQALPPR

SEQ ID NO: 61 - protein, 375 aa, synthetic construct
  source 1..375: note = Fusion protein NYESO1 TCR alpha chain and CD3 zeta chain sequence (NKp30 signal sequence)
MAWMLLLILIMVHPGSCAQKEVEQNSGPLSVPEGAIASLNCTYSDRGSQSFFWYRQYSGKSPELIMFIYSNGDKEDGRFTAQLNKASQYVSLLIRDSQPSDSATYLCAADDKIIFGKGTRLHILPNIQNPDPAVYQLRDSKSSDKSVCLFTDFDSQTNVSQSKDSDVYITDKCVLDMRSMDFKSNSAVAWSNKSDFACANAFNNSIIPEDTFFPSSDVPCDVKLVEKSFETDTNLNFQNLSLCYLLDGILFIYGVILTALFLRVKFSRSADAPAYQQGQNQLYNELNLGRREEYDVLDKRRGRDPEMGGKPQRRKNPQEGLYNELQKDKMAEAYSEIGMKGERRRGKGHDGLYQGLSTATKDTYDALHMQALPPR

SEQ ID NO: 62 - protein, 427 aa, synthetic construct
  source 1..427: note = Fusion protein NYESO1 TCR beta chain and CD3 zeta chain sequence (NKp44 signal sequence, with 9-mer epitope tag)
MAWRALHPLLLLLLLFPGSQADAGVIQSPRHEVTEMGQEVTLRCKPISGHDYLFWYRQTMMRGLELLIYFNNNVPIDDSGMPEDRFSAKMPNASFSTLKIQPSEPRDSAVYFCASSRGGSGYTFGSGTRLTVVEDLNKVFPPEVAVFEPSKAEIAHTQKATLVCLATGFFPDHVELSWWVNGKEVHSGVCTDPQPLKEQPALNDGSGGEVPKDRFSGSGSRYCLSSRLRVSATFWQNPRNHFRCQVQFYGLSENDEWTQDRAKPVTQIVSAEAWGRADCGITSASYHQGVLSALCYLLDGILFIYGVILTALFLRVKFSRSADAPAYQQGQNQLYNELNLGRREEYDVLDKRRGRDPEMGGKPQRRKNPQEGLYNELQKDKMAEAYSEIGMKGERRRGKGHDGLYQGLSTATKDTYDALHMQALPPR

SEQ ID NO: 63 - protein, 378 aa, synthetic construct
  source 1..378: note = Fusion protein NYESO1 TCR alpha chain and CD3 zeta chain sequence (NKp44 signal sequence)
MAWRALHPLLLLLLLFPGSQAQKEVEQNSGPLSVPEGAIASLNCTYSDRGSQSFFWYRQYSGKSPELIMFIYSNGDKEDGRFTAQLNKASQYVSLLIRDSQPSDSATYLCAADDKIIFGKGTRLHILPNIQNPDPAVYQLRDSKSSDKSVCLFTDFDSQTNVSQSKDSDVYITDKCVLDMRSMDFKSNSAVAWSNKSDFACANAFNNSIIPEDTFFPSSDVPCDVKLVEKSFETDTNLNFQNLSLCYLLDGILFIYGVILTALFLRVKFSRSADAPAYQQGQNQLYNELNLGRREEYDVLDKRRGRDPEMGGKPQRRKNPQEGLYNELQKDKMAEAYSEIGMKGERRRGKGHDGLYQGLSTATKDTYDALHMQALPPR

SEQ ID NO: 64 - protein, 425 aa, synthetic construct
  source 1..425: note = Fusion protein NYESO1 TCR beta chain and CD3 zeta chain sequence (TCR beta signal sequence, with 9-mer epitope tag)
MGSWTLCCVSLCILVAKHTDAGVIQSPRHEVTEMGQEVTLRCKPISGHDYLFWYRQTMMRGLELLIYFNNNVPIDDSGMPEDRFSAKMPNASFSTLKIQPSEPRDSAVYFCASSRGGSGYTFGSGTRLTVVEDLNKVFPPEVAVFEPSKAEIAHTQKATLVCLATGFFPDHVELSWWVNGKEVHSGVCTDPQPLKEQPALNDGSGGEVPKDRFSGSGSRYCLSSRLRVSATFWQNPRNHFRCQVQFYGLSENDEWTQDRAKPVTQIVSAEAWGRADCGITSASYHQGVLSALCYLLDGILFIYGVILTALFLRVKFSRSADAPAYQQGQNQLYNELNLGRREEYDVLDKRRGRDPEMGGKPQRRKNPQEGLYNELQKDKMAEAYSEIGMKGERRRGKGHDGLYQGLSTATKDTYDALHMQALPPR

SEQ ID NO: 65 - protein, 378 aa, synthetic construct
  source 1..378: note = Fusion protein NYESO1 TCR alpha chain and CD3 zeta chain sequence (TCR alpha signal sequence)
MKSLRVLLVILWLQLSWVWSQQKEVEQNSGPLSVPEGAIASLNCTYSDRGSQSFFWYRQYSGKSPELIMFIYSNGDKEDGRFTAQLNKASQYVSLLIRDSQPSDSATYLCAADDKIIFGKGTRLHILPNIQNPDPAVYQLRDSKSSDKSVCLFTDFDSQTNVSQSKDSDVYITDKCVLDMRSMDFKSNSAVAWSNKSDFACANAFNNSIIPEDTFFPSSDVPCDVKLVEKSFETDTNLNFQNLSLCYLLDGILFIYGVILTALFLRVKFSRSADAPAYQQGQNQLYNELNLGRREEYDVLDKRRGRDPEMGGKPQRRKNPQEGLYNELQKDKMAEAYSEIGMKGERRRGKGHDGLYQGLSTATKDTYDALHMQALPPR

SEQ ID NO: 66 - DNA, 324 bp, Homo sapiens
  source 1..324: mol_type = other DNA; note = NYESO1 V alpha sequence
cagaaagaggtggaacagaacagcggccctctgtctgtgcctgaaggcgccattgctagcctgaattgcacctactccgaccggggcagccagagcttcttctggtataggcagtacagcggcaagagccccgagctgatcatgtttatctacagcaacggcgacaaagaggacggccggtttacagcccagctgaacaaagccagccagtacgtgtcactgctgattcgggatagccagccaagcgacagcgccacatatctgtgtgccgccgacgacaagatcatcttcggcaagggaaccagactgcacatcctgcctaac

SEQ ID NO: 67 - DNA, 336 bp, Homo sapiens
  source 1..336: mol_type = other DNA; note = NYESO1 V beta sequence
gatgccggcgtgatccagtctcctagacacgaagtgaccgagatgggccaagaagtgaccctgcgctgcaagcctatcagcggccacgattacctgttctggtacagacagaccatgatgagaggcctggaactgctgatctacttcaacaacaacgtgcccatcgacgacagcggcatgcccgaggatagattcagcgccaagatgcccaacgccagctttagcaccctgaagatccagcctagcgagcccagagatagcgccgtgtacttttgcgcctcttccagaggcggcagcggctacacatttggctctggcacaagactgaccgtggtg

SEQ ID NO: 68 - DNA, 345 bp, Homo sapiens
  source 1..345: mol_type = other DNA; note = NYESO1 C alpha sequence
attcagaaccccgatcctgccgtgtaccagctgagagacagcaagagcagcgacaagagcgtgtgcctgttcaccgacttcgacagccagaccaacgtgtcccagagcaaggacagcgacgtgtacatcaccgataagtgcgtgctggatatgcgcagcatggacttcaagagcaacagcgccgtggcctggtccaacaagagcgatttcgcctgcgccaacgccttcaacaatagcattatccccgaggacacattcttccccagctccgatgtgccctgcgacgtgaagctggtggaaaagagcttcgaaaccgacaccaacctgaacttccagaacctgagc

SEQ ID NO: 69 - DNA, 480 bp, synthetic construct
  source 1..480: mol_type = other DNA; note = NYESO1 C beta sequence (with 9-mer epitope tag)
gaagatctgaacaaggtgttccctccagaggtggccgtgttcgagccttctaaggccgagatcgcccacactcagaaagccacactcgtgtgtctggccaccggctttttccccgatcacgtggaactgtcttggtgggtcaacggcaaagaggtgcacagcggcgtctgtaccgatcctcagcctctgaaagagcagcccgctctgaacgatggatctggcggagaggtgcccaaggacagattttctggcagcggcagcagatactgcctgagcagcagactgagagtgtccgccaccttctggcagaaccccagaaaccacttcagatgccaggtgcagttctacggcctgagcgagaacgatgagtggacccaggatagagccaagcctgtgacacagatcgtgtctgccgaagcctggggcagagccgattgtggaattaccagcgccagctaccatcagggcgtgctgtctgcc

SEQ ID NO: 70 - DNA, 1281 bp, synthetic construct
  source 1..1281: mol_type = other DNA; note = Fusion protein NYESO1 TCR beta chain and CD3 zeta chain sequence (NKp46 signal sequence, with 9-mer epitope tag)
atgagcagcaccctgcctgctctgctgtgtgtgggactgtgtctgagccagagaatctctgccgatgccggcgtgatccagtctcctagacacgaagtgaccgagatgggccaagaagtgaccctgcgctgcaagcctatcagcggccacgattacctgttctggtacagacagaccatgatgagaggcctggaactgctgatctacttcaacaacaacgtgcccatcgacgacagcggcatgcccgaggatagattcagcgccaagatgcccaacgccagctttagcaccctgaagatccagcctagcgagcccagagatagcgccgtgtacttttgcgcctcttccagaggcggcagcggctacacatttggctctggcacaagactgaccgtggtggaagatctgaacaaggtgttccctccagaggtggccgtgttcgagccttctaaggccgagatcgcccacactcagaaagccacactcgtgtgtctggccaccggctttttccccgatcacgtggaactgtcttggtgggtcaacggcaaagaggtgcacagcggcgtctgtaccgatcctcagcctctgaaagagcagcccgctctgaacgatggatctggcggagaggtgcccaaggacagattttctggcagcggcagcagatactgcctgagcagcagactgagagtgtccgccaccttctggcagaaccccagaaaccacttcagatgccaggtgcagttctacggcctgagcgagaacgatgagtggacccaggatagagccaagcctgtgacacagatcgtgtctgccgaagcctggggcagagccgattgtggaattaccagcgccagctaccatcagggcgtgctgtctgccctgtgctatctgctggatggcatcctgttcatctacggcgttatcctgacagccctgttcctgagagtgaagttcagcagaagcgccgacgctcctgcttatcagcagggccagaaccagctgtacaacgagctgaacctggggagaagagaagagtacgacgtgctggacaagcggagaggcagagatcctgagatgggcggaaagccccagcggagaaagaatcctcaagagggcctgtataatgagctgcagaaagacaagatggccgaggcctacagcgagatcggaatgaagggcgagcgcagaagaggcaagggacacgatggactgtaccagggcctgagcaccgccaccaaggatacctatgatgccctgcacatgcaggccctgcctccaaga

SEQ ID NO: 71 - DNA, 1134 bp, synthetic construct
  source 1..1134: mol_type = other DNA; note = Fusion protein NYESO1 TCR alpha chain and CD3 zeta chain sequence (NKp46 signal sequence)
atgtctagcacactgcccgcactgctctgcgttggcctgtgtctgtctcagaggatcagcgcccagaaagaggtggaacagaacagcggccctctgtctgtgcctgaaggcgccattgctagcctgaattgcacctactccgaccggggcagccagagcttcttctggtataggcagtacagcggcaagagccccgagctgatcatgtttatctacagcaacggcgacaaagaggacggccggtttacagcccagctgaacaaagccagccagtacgtgtcactgctgattcgggatagccagccaagcgacagcgccacatatctgtgtgccgccgacgacaagatcatcttcggcaagggaaccagactgcacatcctgcctaacattcagaaccccgatcctgccgtgtaccagctgagagacagcaagagcagcgacaagagcgtgtgcctgttcaccgacttcgacagccagaccaacgtgtcccagagcaaggacagcgacgtgtacatcaccgataagtgcgtgctggatatgcgcagcatggacttcaagagcaacagcgccgtggcctggtccaacaagagcgatttcgcctgcgccaacgccttcaacaatagcattatccccgaggacacattcttccccagctccgatgtgccctgcgacgtgaagctggtggaaaagagcttcgaaaccgacaccaacctgaacttccagaacctgagcctgtgttacctgctcgacgggattctctttatctatggcgtgatactgaccgctctgtttctgcgggtcaagttctccagatccgctgacgccccagcataccagcagggacaaaatcagctctataacgaactgaatctcggcaggcgcgaggaatatgacgtcctggataagaggcggggacgcgaccctgaaatgggaggaaaacctcagaggcggaagaacccacaagaaggcctttacaacgaactgcaaaaggataagatggctgaagcttactccgagattggcatgaagggcgaacgtcggagaggaaaaggccacgacggactctatcagggactgtctacagccacaaaggacacatacgacgcactccatatgcaggctctcccacctaga

SEQ ID NO: 72 - DNA, 1362 bp, synthetic construct
  source 1..1362: mol_type = other DNA; note = Fusion protein NYESO1 TCR beta chain, CD3 zeta chain and DAP10 sequence (NKp46 signal se-quence, with 9-mer epitope tag)
atgagcagcaccctgcctgctctgctgtgtgtgggactgtgtctgagccagagaatctctgccgatgccggcgtgatccagtctcctagacacgaagtgaccgagatgggccaagaagtgaccctgcgctgcaagcctatcagcggccacgattacctgttctggtacagacagaccatgatgagaggcctggaactgctgatctacttcaacaacaacgtgcccatcgacgacagcggcatgcccgaggatagattcagcgccaagatgcccaacgccagctttagcaccctgaagatccagcctagcgagcccagagatagcgccgtgtacttttgcgcctcttccagaggcggcagcggctacacatttggctctggcacaagactgaccgtggtggaagatctgaacaaggtgttccctccagaggtggccgtgttcgagccttctaaggccgagatcgcccacactcagaaagccacactcgtgtgtctggccaccggctttttccccgatcacgtggaactgtcttggtgggtcaacggcaaagaggtgcacagcggcgtctgtaccgatcctcagcctctgaaagagcagcccgctctgaacgatggatctggcggagaggtgcccaaggacagattttctggcagcggcagcagatactgcctgagcagcagactgagagtgtccgccaccttctggcagaaccccagaaaccacttcagatgccaggtgcagttctacggcctgagcgagaacgatgagtggacccaggatagagccaagcctgtgacacagatcgtgtctgccgaagcctggggcagagccgattgtggaattaccagcgccagctaccatcagggcgtgctgtctgccctgtgctatctgctggatggcatcctgttcatctacggcgttatcctgacagccctgttcctgagagtgaagttcagcagaagcgccgacgctcctgcttatcagcagggccagaaccagctgtacaacgagctgaacctggggagaagagaagagtacgacgtgctggacaagcggagaggcagagatcctgagatgggcggaaagccccagcggagaaagaatcctcaagagggcctgtataatgagctgcagaaagacaagatggccgaggcctacagcgagatcggaatgaagggcgagcgcagaagaggcaagggacacgatggactgtaccagggcctgagcaccgccaccaaggatacctatgatgccctgcacatgcaggccctgcctccaagaggcggatctctgtgtgcccggcctagaagatctcccgctcaagaggatggcaaggtgtacatcaacatgcccggcagaggt

SEQ ID NO: 73 - DNA, 1134 bp, synthetic construct
  source 1..1134: mol_type = other DNA; note = Fusion protein NYESO1 TCR alpha chain, CD3 zeta chain sequence (NKp46 signal sequence)
atgtctagcacactgcccgcactgctctgcgttggcctgtgtctgtctcagaggatcagcgcccagaaagaagtggaacagaacagcggccctctgagcgttccagaaggcgccattgctagcctgaattgcacctactccgaccggggcagccagagcttcttctggtataggcagtacagcggcaagagccccgagctgatcatgtttatctacagcaacggcgacaaagaggacggccggtttacagcccagctgaacaaagccagccagtacgtgtcactgctgattcgggatagccagccaagcgacagcgccacatatctgtgcgccgctgacgacaagatcatcttcggcaagggcaccagactgcacatcctgcctaacattcagaaccccgatcctgccgtgtaccagctgagagacagcaagagcagcgacaagagcgtgtgcctgttcaccgacttcgacagccagaccaacgtgtcccagagcaaggacagcgacgtgtacattaccgataagtgcgtgctggatatgcgcagcatggacttcaagagcaacagcgccgtggcctggtccaacaagagcgatttcgcctgcgccaacgccttcaacaatagcattatccccgaggacacattcttccccagctccgatgtgccctgcgacgtgaagctggtggaaaagagcttcgaaaccgacaccaacctgaacttccagaacctgagcctgtgttacctgctcgacgggattctctttatctatggcgtgatactgaccgctctgtttctgcgggtcaagttctccagatccgctgacgccccagcataccagcagggacaaaatcagctctataacgaactgaatctcggcaggcgcgaggaatatgacgtcctggataagaggcggggacgcgaccctgaaatgggaggaaaacctcagaggcggaagaacccacaagaaggcctttacaacgaactgcaaaaggataagatggctgaagcttactccgagattggcatgaagggcgaacgtcggagaggaaaaggccacgacggactctatcagggactgtctacagccacaaaggacacatacgacgcactccatatgcaggctctcccacctaga

SEQ ID NO: 74 - DNA, 1215 bp, synthetic construct
  source 1..1215: mol_type = other DNA; note = Fusion protein NYESO1 TCR alpha chain, CD3 zeta chain and DAP10 sequence (NKp46 signal sequence)
atgtctagcacactgcccgcactgctctgcgttggcctgtgtctgtctcagaggatcagcgcccagaaagaagtggaacagaacagcggccctctgagcgttccagaaggcgccattgctagcctgaattgcacctactccgaccggggcagccagagcttcttctggtataggcagtacagcggcaagagccccgagctgatcatgtttatctacagcaacggcgacaaagaggacggccggtttacagcccagctgaacaaagccagccagtacgtgtcactgctgattcgggatagccagccaagcgacagcgccacatatctgtgcgccgctgacgacaagatcatcttcggcaagggcaccagactgcacatcctgcctaacattcagaaccccgatcctgccgtgtaccagctgagagacagcaagagcagcgacaagagcgtgtgcctgttcaccgacttcgacagccagaccaacgtgtcccagagcaaggacagcgacgtgtacattaccgataagtgcgtgctggatatgcgcagcatggacttcaagagcaacagcgccgtggcctggtccaacaagagcgatttcgcctgcgccaacgccttcaacaatagcattatccccgaggacacattcttccccagctccgatgtgccctgcgacgtgaagctggtggaaaagagcttcgaaaccgacaccaacctgaacttccagaacctgagcctgtgttacctgctcgacgggattctctttatctatggcgtgatactgaccgctctgtttctgcgggtcaagttctccagatccgctgacgccccagcataccagcagggacaaaatcagctctataacgaactgaatctcggcaggcgcgaggaatatgacgtcctggataagaggcggggacgcgaccctgaaatgggaggaaaacctcagaggcggaagaacccacaagaaggcctttacaacgaactgcaaaaggataagatggctgaagcttactccgagattggcatgaagggcgaacgtcggagaggaaaaggccacgacggactctatcagggactgtctacagccacaaaggacacatacgacgcactccatatgcaggctctcccacctcgcggtggaagcctttgtgcaagacccagaaggtcccctgcacaagaagatgggaaagtctatatcaatatgcctggcaggggc

SEQ ID NO: 75 - DNA, 63 bp, synthetic construct
  source 1..63: mol_type = other DNA; note = Nkp46 signal sequence 1
atgagcagcaccctgcctgctctgctgtgtgtgggactgtgtctgagccagagaatctctgcc

SEQ ID NO: 76 - DNA, 63 bp, synthetic construct
  source 1..63: mol_type = other DNA; note = Nkp46 signal sequence 2
atgtctagcacactgcccgcactgctctgcgttggcctgtgtctgtctcagaggatcagcgcc

SEQ ID NO: 77 - DNA, 54 bp, synthetic construct
  source 1..54: mol_type = other DNA; note = Nkp30 signal sequence 1
atggcctggatgctgctgctgatcctgatcatggtgcaccctggctcttgtgcc

SEQ ID NO: 78 - DNA, 54 bp, synthetic construct
  source 1..54: mol_type = other DNA; note = Nkp30 signal sequence 2
atggcctggatgctgctgctgatcctgatcatggtgcaccctggcagctgcgcc

SEQ ID NO: 79 - DNA, 63 bp, synthetic construct
  source 1..63: mol_type = other DNA; note = Nkp44 signal sequence 1
atggcctggcgggctctgcatcctttgttgctgctgctcctgctgttccctggctctcaagct

SEQ ID NO: 80 - DNA, 63 bp, synthetic construct
  source 1..63: mol_type = other DNA; note = Nkp44 signal sequence 2
atggcctggcgggctctgcatcctttgttgctgctgctcctgctgttccctggctctcaggcc

SEQ ID NO: 81 - DNA, 57 bp, synthetic construct
  source 1..57: mol_type = other DNA; note = TCR beta signal sequence
atgggcagctggaccctgtgctgtgtgtccctgtgtatcctggtggccaagcacaca

SEQ ID NO: 82 - DNA, 63 bp, synthetic construct
  source 1..63: mol_type = other DNA; note = TCR alpha signal sequence
atgaagtccctgcgggtgctgctggttatcctgtggctgcagctgagctgggtctggtcccag

SEQ ID NO: 83 - DNA, 402 bp, synthetic construct
  source 1..402: mol_type = other DNA; note = CD3 zeta sequence 1
ctgtgctatctgctggatggcatcctgttcatctacggcgttatcctgacagccctgttcctgagagtgaagttcagcagaagcgccgacgctcctgcttatcagcagggccagaaccagctgtacaacgagctgaacctggggagaagagaagagtacgacgtgctggacaagcggagaggcagagatcctgagatgggcggaaagccccagcggagaaagaatcctcaagagggcctgtataatgagctgcagaaagacaagatggccgaggcctacagcgagatcggaatgaagggcgagcgcagaagaggcaagggacacgatggactgtaccagggcctgagcaccgccaccaaggatacctatgatgccctgcacatgcaggccctgcctccaaga

SEQ ID NO: 84 - DNA, 402 bp, synthetic construct
  source 1..402: mol_type = other DNA; note = CD3 zeta sequence 2
ctgtgttacctgctcgacgggattctctttatctatggcgtgatactgaccgctctgtttctgcgggtcaagttctccagatccgctgacgccccagcataccagcagggacaaaatcagctctataacgaactgaatctcggcaggcgcgaggaatatgacgtcctggataagaggcggggacgcgaccctgaaatgggaggaaaacctcagaggcggaagaacccacaagaaggcctttacaacgaactgcaaaaggataagatggctgaagcttactccgagattggcatgaagggcgaacgtcggagaggaaaaggccacgacggactctatcagggactgtctacagccacaaaggacacatacgacgcactccatatgcaggctctcccacctaga

SEQ ID NO: 85 - DNA, 72 bp, synthetic construct
  source 1..72: mol_type = other DNA; note = DAP10 sequence 1
ctgtgtgcccggcctagaagatctcccgctcaagaggatggcaaggtgtacatcaacatgcccggcagaggt

SEQ ID NO: 86 - DNA, 72 bp, synthetic construct
  source 1..72: mol_type = other DNA; note = DAP10 seqeuence 2
ctttgtgcaagacccagaaggtcccctgcacaagaagatgggaaagtctatatcaatatgcctggcaggggc

SEQ ID NO: 87 - DNA, 1272 bp, synthetic construct
  source 1..1272: mol_type = other DNA; note = Fusion protein NYESO1 TCR beta chain and CD3 zeta chain sequence (NKp30 signal sequence, with 9-mer epitope tag)
atggcctggatgctgctgctgatcctgatcatggtgcaccctggctcttgtgccgatgccggcgttatccagtctcctagacacgaagtgaccgagatgggccaagaagtgaccctgcgctgcaagcctatcagcggccacgattacctgttctggtacagacagaccatgatgagaggcctggaactgctgatctacttcaacaacaacgtgcccatcgacgacagcggcatgcccgaggatagattcagcgccaagatgcccaacgccagcttcagcaccctgaagatccagcctagcgagcccagagatagcgccgtgtacttttgcgcctcttccagaggcggcagcggctacacatttggctctggcacaagactgaccgtggtggaagatctgaacaaggtgttccctccagaggtggccgtgttcgagccttctaaggccgagattgcccacacacagaaagccacactcgtgtgcctggccaccggctttttccccgatcacgtggaactgtcttggtgggtcaacggcaaagaggtgcacagcggcgtctgtaccgatcctcagcctctgaaagagcagcccgctctgaacgatggatctggcggagaggtgcccaaggacagattttctggcagcggcagcagatactgcctgagcagcagactgagagtgtccgccaccttctggcagaaccccagaaaccacttcagatgccaggtgcagttctacggcctgagcgagaacgatgagtggacccaggatagagccaagcctgtgacacagatcgtgtctgccgaagcctggggcagagccgattgtggaattaccagcgccagctaccatcagggcgtgctgtctgccctgtgctatctgctggatggcatcctgttcatctacggcgtgatcctgacagccctgttcctgagagtgaagttcagcagaagcgccgacgctcctgcttatcagcagggccagaaccagctgtacaacgagctgaacctggggagaagagaagagtacgacgtgctggacaagcggagaggcagagatcctgagatgggcggaaagccccagcggagaaagaatcctcaagagggcctgtataatgagctgcagaaagacaagatggccgaggcctacagcgagatcggaatgaagggcgagcgcagaagaggcaagggacacgatggactgtaccagggcctgagcaccgccaccaaggatacctatgatgccctgcacatgcaggccctgcctccaaga

SEQ ID NO: 88 - DNA, 1125 bp, synthetic construct
  source 1..1125: mol_type = other DNA; note = Fusion protein NYESO1 TCR alpha chain and CD3 zeta chain sequence (NKp30 signal sequence)
atggcctggatgctgctgctgatcctgatcatggtgcaccctggcagctgcgcccagaaagaggtggaacagaatagcggccctctgagcgttccagaaggcgctatcgccagcctgaactgcacctacagcgatagaggcagccagagcttcttctggtacagacagtacagcggcaagagccccgagctgatcatgttcatctacagcaacggcgacaaagaggacggccggtttacagcccagctgaacaaggccagccagtacgtgtccctgctgatcagagatagccagcctagcgacagcgccacctatctgtgtgccgccgacgacaagatcatcttcggcaagggcaccagactgcacatcctgcctaacattcagaaccccgatcctgccgtgtaccagctgagagacagcaagagcagcgacaagagcgtgtgcctgttcaccgacttcgacagccagaccaacgtgtcccagagcaaggacagcgacgtgtacatcaccgataagtgcgtgctggacatgcggagcatggacttcaagagcaacagcgccgtggcctggtccaacaagagcgatttcgcctgcgccaacgccttcaacaacagcattatccccgaggacacattcttccccagctccgatgtgccctgcgacgtgaagctggtggaaaagagcttcgagacagacaccaacctgaacttccagaacctgagcctgtgctacctgctggacggcatcctgtttatctacggcgtgatcctgacagccctgttcctgagagtgaagttcagcagaagcgccgacgctcctgcttaccagcagggccagaaccagctgtacaacgagctgaacctggggagaagagaagagtacgacgtgctggataagcgcagaggcagagatcctgagatgggcggaaagccccagcggagaaagaatcctcaagagggcctgtataatgagctgcagaaagacaagatggccgaggcctactccgagatcggaatgaagggcgagcgcagaagaggcaagggacacgatggactgtaccagggcctgagcaccgccaccaaggatacctatgatgccctgcacatgcaggccctgcctccaaga

SEQ ID NO: 89 - DNA, 1281 bp, synthetic construct
  source 1..1281: mol_type = other DNA; note = Fusion protein NYESO1 TCR beta chain and CD3 zeta chain sequence (NKp44 signal sequence, with 9-mer epitope tag)
atggcctggcgggctctgcatcctttgttgctgctgctcctgctgttccctggctctcaagctgatgccggcgtgatccagtctcctagacacgaagtgaccgagatgggccaagaagtgaccctgcgctgcaagcctatcagcggccacgattacctgttctggtacagacagaccatgatgagaggcctggaactgctgatctacttcaacaacaacgtgcccatcgacgacagcggcatgcccgaggatagattcagcgccaagatgcccaacgccagcttcagcaccctgaagatccagcctagcgagcccagagatagcgccgtgtacttttgcgcctcttccagaggcggcagcggctacacatttggctctggcacaagactgaccgtggtggaagatctgaacaaggtgttccctccagaggtggccgtgttcgagccttctaaggccgagattgcccacacacagaaagccacactcgtgtgcctggccaccggctttttccccgatcacgtggaactgtcttggtgggtcaacggcaaagaggtgcacagcggcgtctgtaccgatcctcagcctctgaaagagcagcccgctctgaacgatggatctggcggagaggtgcccaaggacagattttctggcagcggcagcagatactgcctgagcagcagactgagagtgtccgccaccttctggcagaaccccagaaaccacttcagatgccaggtgcagttctacggcctgagcgagaacgatgagtggacccaggatagagccaagcctgtgacacagatcgtgtctgccgaagcctggggcagagccgattgtggaattaccagcgccagctaccatcagggcgtgctgtctgccctgtgctatctgctggatggcatcctgttcatctacggcgttatcctgacagccctgttcctgagagtgaagttcagcagaagcgccgacgctcctgcttatcagcagggccagaaccagctgtacaacgagctgaacctggggagaagagaagagtacgacgtgctggacaagcggagaggcagagatcctgagatgggcggaaagccccagcggagaaagaatcctcaagagggcctgtataatgagctgcagaaagacaagatggccgaggcctacagcgagatcggaatgaagggcgagcgcagaagaggcaagggacacgatggactgtaccagggcctgagcaccgccaccaaggatacctatgatgccctgcacatgcaggccctgcctccaaga

SEQ ID NO: 90 - DNA, 1134 bp, synthetic construct
  source 1..1134: mol_type = other DNA; note = Fusion protein NYESO1 TCR alpha chain and CD3 zeta chain sequence (NKp44 signal sequence)
atggcctggcgggctctgcatcctttgttgctgctgctcctgctgttccctggctctcaggcccagaaagaggtggaacagaatagcggccctctgagcgttccagaaggcgctatcgccagcctgaactgcacctacagcgatagaggcagccagagcttcttctggtacagacagtacagcggcaagagccccgagctgatcatgttcatctacagcaacggcgacaaagaggacggccggtttacagcccagctgaacaaggccagccagtacgtgtccctgctgatcagagatagccagcctagcgacagcgccacctatctgtgtgccgccgacgacaagatcatcttcggcaagggcaccagactgcacatcctgcctaacattcagaaccccgatcctgccgtgtaccagctgagagacagcaagtccagcgacaagagcgtgtgcctgttcaccgacttcgacagccagaccaacgtgtcccagagcaaggacagcgacgtgtacatcaccgataagtgcgtgctggacatgcggagcatggacttcaagagcaacagcgccgtggcctggtccaacaagagcgatttcgcctgcgccaacgccttcaacaacagcattatccccgaggacacattcttccccagctccgatgtgccctgcgacgtgaagctggtggaaaagagcttcgagacagacaccaacctgaacttccagaacctgagcctgtgctacctgctggacggcatcctgtttatctacggcgtgatcctgacagccctgttcctgagagtgaagttcagcagaagcgccgacgctcctgcttaccagcagggccagaaccagctgtacaacgagctgaacctggggagaagagaagagtacgacgtgctggataagcgcagaggcagagatcctgagatgggcggaaagccccagcggagaaagaatcctcaagagggcctgtataatgagctgcagaaagacaagatggccgaggcctactccgagatcggaatgaagggcgagcgcagaagaggcaagggacacgatggactgtaccagggcctgagcaccgccaccaaggatacctatgatgccctgcacatgcaggccctgcctccaaga

SEQ ID NO: 91 - DNA, 1275 bp, synthetic construct
  source 1..1275: mol_type = other DNA; note = Fusion protein NYESO1 TCR beta chain and CD3 zeta chain sequence (TCR beta signal sequence, with 9-mer epitope tag)
atgggcagctggaccctgtgctgtgtgtccctgtgtatcctggtggccaagcacacagatgccggcgtgatccagtctcctagacacgaagtgaccgagatgggccaagaagtgaccctgcgctgcaagcctatcagcggccacgattacctgttctggtacagacagaccatgatgagaggcctggaactgctgatctacttcaacaacaacgtgcccatcgacgacagcggcatgcccgaggatagattcagcgccaagatgcccaacgccagcttcagcaccctgaagatccagcctagcgagcccagagatagcgccgtgtacttttgcgcctcttccagaggcggcagcggctacacatttggctctggcacaagactgaccgtggtggaagatctgaacaaggtgttccctccagaggtggccgtgttcgagccttctaaggccgagattgcccacacacagaaagccacactcgtgtgcctggctaccggcttctttcccgatcacgtggaactgtcttggtgggtcaacggcaaagaggtgcacagcggcgtctgtaccgatcctcagcctctgaaagagcagcccgctctgaacgatggatctggcggagaggtgcccaaggacagattttctggcagcggcagcagatactgcctgagcagcagactgagagtgtccgccaccttctggcagaaccccagaaaccacttcagatgccaggtgcagttctacggcctgagcgagaacgatgagtggacccaggatagagccaagcctgtgacacagatcgtgtctgccgaagcctggggcagagccgattgtggaattaccagcgccagctaccatcagggcgtgctgagcgctctgtgctatctgctggatggcatcctgttcatctacggcgttatcctgacagccctgttcctgagagtgaagttcagcagaagcgccgacgctcctgcttatcagcagggccagaaccagctgtacaacgagctgaacctggggagaagagaagagtacgacgtgctggacaagcggagaggcagagatcctgagatgggcggaaagccccagcggagaaagaatcctcaagagggcctgtataatgagctgcagaaagacaagatggccgaggcctacagcgagatcggaatgaagggcgagcgcagaagaggcaagggacacgatggactgtaccagggcctgagcaccgccaccaaggacacatatgatgccctgcacatgcaggccctgcctccaaga

SEQ ID NO: 92 - DNA, 1137 bp, synthetic construct
  source 1..1137: mol_type = other DNA; note = Fusion protein NYESO1 TCR alpha chain and CD3 zeta chain sequence (TCR alpha signal sequence)
atgaagtccctgcgggtgctgctggttatcctgtggctgcagctgagctgggtctggtcccagcagaaagaggtggaacagaacagcggccctctgtctgttcctgaaggcgctatcgccagcctgaactgcacctacagcgatagaggcagccagagcttcttctggtacagacagtacagcggcaagagccccgagctgatcatgttcatctacagcaacggcgacaaagaggacggccggtttacagcccagctgaacaaggccagccagtacgtgtccctgctgatcagagatagccagcctagcgacagcgccacctatctgtgtgccgccgacgacaagatcatcttcggcaagggcaccagactgcacatcctgcctaacattcagaaccccgatcctgccgtgtaccagctgagagacagcaagagcagcgacaagagcgtgtgcctgttcaccgacttcgacagccagaccaacgtgtcccagagcaaggacagcgacgtgtacatcaccgataagtgcgtgctggacatgcggagcatggacttcaagagcaacagcgccgtggcctggtccaacaagagcgatttcgcctgcgccaacgccttcaacaacagcattatccccgaggacacattcttccccagctccgatgtgccctgcgacgtgaagctggtggaaaagagcttcgagacagacaccaacctgaacttccagaacctgagcctgtgctacctgctggacggcatcctgtttatctacggcgtgatcctgacagccctgtttctgagagtgaagttcagcagaagcgccgacgctcctgcttaccagcagggccagaaccagctgtacaacgagctgaacctggggagaagagaagagtacgacgtgctggataagcgcagaggcagagatcctgagatgggcggaaagccccagcggagaaagaatcctcaagagggcctgtataatgagctgcagaaagacaagatggccgaggcctactccgagatcggaatgaagggcgagcgcagaagaggcaagggacacgatggactgtaccagggcctgagcaccgccaccaaggatacctatgatgccctgcacatgcaggccctgcctccaagataa

SEQ ID NO: 93 - protein, 16 aa, Homo sapiens
  source 1..16: note = CD16A signal sequence
MWQLLLPTALLLLVSA

SEQ ID NO: 94 - DNA, 48 bp, synthetic construct
  source 1..48: mol_type = other DNA; note = CD16A signal sequence
atgtggcaactgctgctgcctacagctctgctgcttctggtgtctgcc